European Patent Specification EP 4 082 554 B1, published February 26, 2025. Title: COMPOSITION FOR USE IN INHIBITING LIPOFUSCIN ACCUMULATION OR REMOVING LIPOFUSCIN. Applicant: AMOREPACIFIC CORPORATION. The sequence listing filed with the application follows.

SEQUENCE LISTING (3 sequences)

SEQ ID NO: 1 - DNA, 1198 bp, Unknown
  Chryseobacterium camelliae Dolsongi-HT1
agctagggtgggtacggattattgggtttaagggtccgtaggcggatgtgtaagtcagtggtgaaatctcacagcttaactgtgaaactgccattgatactgcatgtcttgagtaaggtagaagtggctggaataagtagtgtagcggtgaaatgcatagatattacttagaacaccaattgcgaaggcaggtcactatgtcttaactgacgctgatggacgaaagcgtggggagcgaacaggattagataccctggtagtccacgccgtaaacgatgctaactcgtttttgggttttcggattcagagactaagcgaaagtgataagttagccacctggggagtacgttcgcaagaatgaaactcaaaggaattgacgggggcccgcacaagcggtggattatgtggtttaattcgatgatacgcgaggaaccttaccaaggcttaaatgggaattgatcggtttagaaatagaccttccttcgggcaattttcaaggtgctgcatggttgtcgtcagctcgtgccgtgaggtgttaggttaagtcctgcaacgagcgcaacccctgttactagttgctaccattaagttgaggactctagtaagactgcctacgcaagtagagaggaaggtggggatgacgtcaaatcatcacggcccttacgccttgggccacacacgtaatacaatggcaggtacagagggcagctacacagcgatgtgatgcgaatctcgaaagcctgtctcagttcggattggagtctgcaactcgactctatgaagctggaatcgctagtaatcgcgcatcagccatggcgcggtgaatacgttcccgggccttgtacacaccgcccgtcaagccatggaagtctggggtacctgaagtcggtgaccgtaaaaggagctgcctagggtaaaacaggtaactagggctaatcgtacaggggaaaccctaaaagtttaaccaggaaccggtagaaggtgttaaggatagagtgtatatctgttttgtatatgttgtatttatctagtgtatctgagataatggatagataacgctcgaactggcactacactagtgagagatattagtattcttatatattaagtctctattgagatatcataatcgtggataaagacttgacagcggcgagagcctggatagcggagtggtgttagctatgagtgtataatc

SEQ ID NO: 2 - DNA, 20 bp, Artificial Sequence
  27F primer
agagtttgatcmtggctcag

SEQ ID NO: 3 - DNA, 22 bp, Artificial Sequence
  1492R primer
tacggytaccttgttacgactt